European Patent Specification EP 3 845 644 B1, published April 24, 2024. Title: NOVEL HUMAN SERUM ALBUMIN MUTANT. Applicant: JCR Pharmaceuticals Co., Ltd. The sequence listing filed with the application follows.

SEQUENCE LISTING (45 sequences)

SEQ ID NO: 1 - protein, 585 aa, Homo sapiens [sequence omitted]

SEQ ID NO: 2 - protein, 586 aa, Homo sapiens
RDAHKSEVAHRFKDLGEENFKALVLIAFAQYLQQCPFEDHVKLVNEVTEFAKTCVADESAENCDKSLHTLFGDKLCTVATLRETYGEMADCCAKQEPERNECFLQHKDDNPNLPRLVRPEVDVMCTAFHDNEETFLKKYLYEIARRHPYFYAPELLFFAKRYKAAFTECCQAADKAACLLPKLDELRDEGKASSAKQRLKCASLQKFGERAFKAWAVARLSQRFPKAEFAEVSKLVTDLTKVHTECCHGDLLECADDRADLAKYICENQDSISSKLKECCEKPLLEKSHCIAEVENDEMPADLPSLAADFVESKDVCKNYTEAKDVFLGMFLYEYARRHPDYSVVLLLRLAKTYETTLEKCCAAADPHECYAKVFDEFKPLVEEPQNLIKQNCELFEQLGEYKFQNALLVRYTKKVPQVSTPTLVEVSRNLGKVGSKCCKHPEAKRMPCAEDYLSVVLNQLCVLHEKTPVSDRVTKCCTESLVNRRPCFSALEVDETYVPKEFNAETFTFHADICTLSEKERQIKKQTALVELVKHKPKATKEQLKAVMDDFAAFVEKCCKADDKETCFAEEGKKLVAASQAALGL

SEQ ID NO: 3 - protein, 585 aa, Artificial Sequence
  Human serum albumin mutant (A320T)
DAHKSEVAHRFKDLGEENFKALVLIAFAQYLQQCPFEDHVKLVNEVTEFAKTCVADESAENCDKSLHTLFGDKLCTVATLRETYGEMADCCAKQEPERNECFLQHKDDNPNLPRLVRPEVDVMCTAFHDNEETFLKKYLYEIARRHPYFYAPELLFFAKRYKAAFTECCQAADKAACLLPKLDELRDEGKASSAKQRLKCASLQKFGERAFKAWAVARLSQRFPKAEFAEVSKLVTDLTKVHTECCHGDLLECADDRADLAKYICENQDSISSKLKECCEKPLLEKSHCIAEVENDEMPADLPSLAADFVESKDVCKNYTEAKDVFLGMFLYEYARRHPDYSVVLLLRLAKTYETTLEKCCAAADPHECYAKVFDEFKPLVEEPQNLIKQNCELFEQLGEYKFQNALLVRYTKKVPQVSTPTLVEVSRNLGKVGSKCCKHPEAKRMPCAEDYLSVVLNQLCVLHEKTPVSDRVTKCCTESLVNRRPCFSALEVDETYVPKEFNAETFTFHADICTLSEKERQIKKQTALVELVKHKPKATKEQLKAVMDDFAAFVEKCCKADDKETCFAEEGKKLVAASQAALGL

SEQ ID NO: 4 - protein, 5 aa, Artificial Sequence
  Example of linker
GGGGS

SEQ ID NO: 5 - protein, 6 aa, Artificial Sequence
  Example of linker
GGGGGS

SEQ ID NO: 6 - protein, 5 aa, Artificial Sequence
  Example of linker
SGGGG

SEQ ID NO: 7 - DNA, 23 bp, Murine encephalomyocardinitis virus
atgataatatggccacaaccatg

SEQ ID NO: 8 - DNA, 23 bp, Artificial Sequence
  Partial sequence of IRES from mutant type murine encephalomyocardinitis virus
atgataagcttgccacaaccatg

SEQ ID NO: 9 - protein, 191 aa, Homo sapiens [sequence omitted]

SEQ ID NO: 10 - protein, 176 aa, Homo sapiens
FPTIPLSRLFDNAMLRAHRLHQLAFDTYQEFNPQTSLCFSESIPTPSNREETQQKSNLELLRISLLLIQSWLEPVQFLRSVFANSLVYGASDSNVYDLLKDLEEGIQTLMGRLEDGSPRTGQIFKQTYSKFDTNSHNDDALLKNYGLLYCFRKDMDKVETFLRIVQCRSVEGSCGF

SEQ ID NO: 11 - protein, 776 aa, Artificial Sequence
  22KhGH-mHSA
FPTIPLSRLFDNAMLRAHRLHQLAFDTYQEFEEAYIPKEQKYSFLQNPQTSLCFSESIPTPSNREETQQKSNLELLRISLLLIQSWLEPVQFLRSVFANSLVYGASDSNVYDLLKDLEEGIQTLMGRLEDGSPRTGQIFKQTYSKFDTNSHNDDALLKNYGLLYCFRKDMDKVETFLRIVQCRSVEGSCGFDAHKSEVAHRFKDLGEENFKALVLIAFAQYLQQCPFEDHVKLVNEVTEFAKTCVADESAENCDKSLHTLFGDKLCTVATLRETYGEMADCCAKQEPERNECFLQHKDDNPNLPRLVRPEVDVMCTAFHDNEETFLKKYLYEIARRHPYFYAPELLFFAKRYKAAFTECCQAADKAACLLPKLDELRDEGKASSAKQRLKCASLQKFGERAFKAWAVARLSQRFPKAEFAEVSKLVTDLTKVHTECCHGDLLECADDRADLAKYICENQDSISSKLKECCEKPLLEKSHCIAEVENDEMPADLPSLAADFVESKDVCKNYTEAKDVFLGMFLYEYARRHPDYSVVLLLRLAKTYETTLEKCCAAADPHECYAKVFDEFKPLVEEPQNLIKQNCELFEQLGEYKFQNALLVRYTKKVPQVSTPTLVEVSRNLGKVGSKCCKHPEAKRMPCAEDYLSVVLNQLCVLHEKTPVSDRVTKCCTESLVNRRPCFSALEVDETYVPKEFNAETFTFHADICTLSEKERQIKKQTALVELVKHKPKATKEQLKAVMDDFAAFVEKCCKADDKETCFAEEGKKLVAASQAALGL

SEQ ID NO: 12 - protein, 761 aa, Artificial Sequence
  20KhGH-mHSA
FPTIPLSRLFDNAMLRAHRLHQLAFDTYQEFNPQTSLCFSESIPTPSNREETQQKSNLELLRISLLLIQSWLEPVQFLRSVFANSLVYGASDSNVYDLLKDLEEGIQTLMGRLEDGSPRTGQIFKQTYSKFDTNSHNDDALLKNYGLLYCFRKDMDKVETFLRIVQCRSVEGSCGFDAHKSEVAHRFKDLGEENFKALVLIAFAQYLQQCPFEDHVKLVNEVTEFAKTCVADESAENCDKSLHTLFGDKLCTVATLRETYGEMADCCAKQEPERNECFLQHKDDNPNLPRLVRPEVDVMCTAFHDNEETFLKKYLYEIARRHPYFYAPELLFFAKRYKAAFTECCQAADKAACLLPKLDELRDEGKASSAKQRLKCASLQKFGERAFKAWAVARLSQRFPKAEFAEVSKLVTDLTKVHTECCHGDLLECADDRADLAKYICENQDSISSKLKECCEKPLLEKSHCIAEVENDEMPADLPSLAADFVESKDVCKNYTEAKDVFLGMFLYEYARRHPDYSVVLLLRLAKTYETTLEKCCAAADPHECYAKVFDEFKPLVEEPQNLIKQNCELFEQLGEYKFQNALLVRYTKKVPQVSTPTLVEVSRNLGKVGSKCCKHPEAKRMPCAEDYLSVVLNQLCVLHEKTPVSDRVTKCCTESLVNRRPCFSALEVDETYVPKEFNAETFTFHADICTLSEKERQIKKQTALVELVKHKPKATKEQLKAVMDDFAAFVEKCCKADDKETCFAEEGKKLVAASQAALGL

SEQ ID NO: 13 - DNA, 20 bp, Artificial Sequence
  Primer Hyg-Sfi5', synthetic
gaggccgcctcggcctctga

SEQ ID NO: 14 - DNA, 29 bp, Artificial Sequence
  Primer Hyg-BstX3', synthetic
aaccatcgtgatgggtgctattcctttgc

SEQ ID NO: 15 - DNA, 2216 bp, Artificial Sequence
  IRES-Hygr-mPGKpA, synthetic
ctcgaggaattcactccttcaggtgcaggcttgcctatcagaaggtggtggctggtgtggccaactggctcacaaataccactgagatcgacggtatcgataagcttgatatcgaattccgccccccccccctctccctcccccccccctaacgttactggccgaagccgcttggaataaggccggtgtgcgtttgtctatatgttattttccaccatattgccgtcttttggcaatgtgagggcccggaaacctggccctgtcttcttgacgagcattcctaggggtctttcccctctcgccaaaggaatgcaaggtctgttgaatgtcgtgaaggaagcagttcctctggaagcttcttgaagacaaacaacgtctgtagcgaccctttgcaggcagcggaaccccccacctggcgacaggtgcctctgcggccaaaagccacgtgtataagatacacctgcaaaggcggcacaaccccagtgccacgttgtgagttggatagttgtggaaagagtcaaatggctctcctcaagcgtattcaacaaggggctgaaggatgcccagaaggtaccccattgtatgggatctgatctggggcctcggtgcacatgctttacatgtgtttagtcgaggttaaaaaaacgtctaggccccccgaaccacggggacgtggttttcctttgaaaaacacgatgataatatggccacaaccatgaaaaagcctgaactcaccgcgacgtctgtcgagaagtttctgatcgaaaagttcgacagcgtctccgacctgatgcagctctcggagggcgaagaatctcgtgctttcagcttcgatgtaggagggcgtggatatgtcctgcgggtaaatagctgcgccgatggtttctacaaagatcgttatgttcatcggcactttgcatcggccgcgctcccgattccggaagtgcttgacattggggaattcagcgagagcctgacctattgcatctcccgccgtgcacagggtgtcacgttgcaagacctgcctgaaaccgaactgcccgctgttctgcagccggtcgcggaggccatggatgcgatcgctgcggccgatcttagccagacgagcgggttcggcccattcggaccgcaaggaatcggtcaatacactacgtggcgtgatttcatatgcgcgattgctgatccccatgtgtatcactggcaaactgtgatggacgacaccgtcagtgcgtccgtcgcgcaggctctcgatgagctgatgctttgggccgaggactgccccgaagtccggcacctcgtgcacgcggatttcggctccaacaatgtcctgacggacaatggccgcataacagcggtcattgactggagcgaggcgatgttcggggattcccaatacgaggtcgccaacatcttcttctggaggccgtggttggcttgtatggagcagcagacgcgctacttcgagcggaggcatccggagcttgcaggatcgccgcggctccgggcgtatatgctccgcattggtcttgaccaactctatcagagcttggttgacggcaatttcgatgatgcagcttgggcgcagggtcgatgcgacgcaatcgtccgatccggagccgggactgtcgggcgtacacaaatcgcccgcagaagcgcggccgtctggaccgatggctgtgtagaagtactcgccgatagtggaaaccgacgccccagcactcgtccgagggcaaaggaatagtcgagaaattgatgatctattaagcaataaagacgtccactaaaatggaagtttttcctgtcatactttgttaagaagggtgagaacagagtacctacattttgaatggaaggattggagctacgggggtgggggtggggtgggattagataaatgcctgctctttactgaaggctctttactattgctttatgataatgtttcatagttggatatcataatttaaacaagcaaaaccaaattaagggccagctcattcctccactcacgatctatagatccactagcttggcgtaatcatggtcatagctgtttcctgtgtgaaattgttatccgctcacaattccacacaacatacgagccggaagcataaagtgtaaagcctggggtgcctaatgagtgagctaactcacattaattgcgttgcgctcactgcccgctttccagtcgggaaacctgtcgtgccagcggatcc

SEQ ID NO: 16 - protein, 341 aa, Artificial Sequence
  Amino acid sequence corresponding to hygromycin resistance gen
MKKPELTATSVEKFLIEKFDSVSDLMQLSEGEESRAFSFDVGGRGYVLRVNSCADGFYKDRYVHRHFASAALPIPEVLDIGEFSESLTYCISRRAQGVTLQDLPETELPAVLQPVAEAMDAIAAADLSQTSGFGPFGPQGIGQYTTWRDFICAIADPHVYHWQTVMDDTVSASVAQALDELMLWAEDCPEVRHLVHADFGSNNVLTDNGRITAVIDWSEAMFGDSQYEVANIFFWRPWLACMEQQTRYFERRHPELAGSPRLRAYMLRIGLDQLYQSLVDGNFDDAAWAQGRCDAIVRSGAGTVGRTQIARRSAAVWTDGCVEVLADSGNRRPSTRPRAKE

SEQ ID NO: 17 - DNA, 53 bp, Artificial Sequence
  Primer IRES5', synthetic
caactcgagcggccgccccccccccctctccctcccccccccctaacgttact

SEQ ID NO: 18 - DNA, 22 bp, Artificial Sequence
  Primer IRES3', synthetic
caagaagcttccagaggaactg

SEQ ID NO: 19 - DNA, 30 bp, Artificial Sequence
  Primer mPGKP5', synthetic
gcgagatcttaccgggtaggggaggcgctt

SEQ ID NO: 20 - DNA, 30 bp, Artificial Sequence
  Primer mPGKP3', synthetic
gaggaattcgatgatcggtcgaaaggcccg

SEQ ID NO: 21 - DNA, 532 bp, Artificial Sequence
  mPGKp, synthetic
gcgagatcttaccgggtaggggaggcgcttttcccaaggcagtctggagcatgcgctttagcagccccgctgggcacttggcgctacacaagtggcctctggcctcgcacacattccacatccaccggtaggcgccaaccggctccgttctttggtggccccttcgcgccaccttctactcctcccctagtcaggaagttcccccccgccccgcagctcgcgtcgtgcaggacgtgacaaatggaagtagcacgtctcactagtctcgtgcagatggacagcaccgctgagcaatggaagcgggtaggcctttggggcagcggccaatagcagctttgctccttcgctttctgggctcagaggctgggaaggggtgggtccgggggcgggctcaggggcgggctcaggggcggggcgggcgcccgaaggtcctccggaggcccggcattctgcacgcttcaaaagcgcacgtctgccgcgctgttctcctcttcctcatctccgggcctttcgaccgatcatcgaattcctc

SEQ ID NO: 22 - DNA, 36 bp, Artificial Sequence
  Primer GS5', synthetic
aatatggccacaaccatggcgacctcagcaagttcc

SEQ ID NO: 23 - DNA, 38 bp, Artificial Sequence
  Primer GS3', synthetic
ggaggatccctcgagttagtttttgtattggaagggct

SEQ ID NO: 24 - DNA, 28 bp, Artificial Sequence
  Primer puro5', synthetic
gcttaagatgaccgagtacaagcccacg

SEQ ID NO: 25 - DNA, 30 bp, Artificial Sequence
  Primer puro3', synthetic
cccatcgtgatggtcaggcaccgggcttgc

SEQ ID NO: 26 - DNA, 620 bp, Artificial Sequence
  Sequence containing puromycin resistance gene, synthetic
gcttaagatgaccgagtacaagcccacggtgcgcctcgccacccgcgacgacgtccccagggccgtacgcaccctcgccgccgcgttcgccgactaccccgccacgcgccacaccgtcgatccggaccgccacatcgagcgggtcaccgagctgcaagaactcttcctcacgcgcgtcgggctcgacatcggcaaggtgtgggtcgcggacgacggcgccgcggtggcggtctggaccacgccggagagcgtcgaagcgggggcggtgttcgccgagatcggcccgcgcatggccgagttgagcggttcccggctggccgcgcagcaacagatggaaggcctcctggcgccgcaccggcccaaggagcccgcgtggttcctggccaccgtcggcgtctcgcccgaccaccagggcaagggtctgggcagcgccgtcgtgctccccggagtggaggcggccgagcgcgccggggtgcccgccttcctggagacctccgcgccccgcaacctccccttctacgagcggctcggcttcaccgtcaccgccgacgtcgaggtgcccgaaggaccgcgcacctggtgcatgacccgcaagcccggtgcctgaccatcacgatggg

SEQ ID NO: 27 - protein, 199 aa, Artificial Sequence
  Amino acid sequence corresponding to puromycin resistance gene
MTEYKPTVRLATRDDVPRAVRTLAAAFADYPATRHTVDPDRHIERVTELQELFLTRVGLDIGKVWVADDGAAVAVWTTPESVEAGAVFAEIGPRMAELSGSRLAAQQQMEGLLAPHRPKEPAWFLATVGVSPDHQGKGLGSAVVLPGVEAAERAGVPAFLETSAPRNLPFYERLGFTVTADVEVPEGPRTWCMTRKPGA

SEQ ID NO: 28 - DNA, 44 bp, Artificial Sequence
  Primer SV40polyA5', synthetic
caacaagcggccgccctcgagttccctttagtgagggttaatgc

SEQ ID NO: 29 - DNA, 24 bp, Artificial Sequence
  Primer SV40polyA3', synthetic
cccctgaacctgaaacataaaatg

SEQ ID NO: 30 - DNA, 25 bp, Artificial Sequence
  Primer mIRES-GS5', synthetic
acacgatgataagcttgccacaacc

SEQ ID NO: 31 - DNA, 21 bp, Artificial Sequence
  Primer mIRES-GS3', synthetic
ctccacgatatccctgccata

SEQ ID NO: 32 - protein, 776 aa, Artificial Sequence
  HSA-22KhGH, mature
DAHKSEVAHRFKDLGEENFKALVLIAFAQYLQQCPFEDHVKLVNEVTEFAKTCVADESAENCDKSLHTLFGDKLCTVATLRETYGEMADCCAKQEPERNECFLQHKDDNPNLPRLVRPEVDVMCTAFHDNEETFLKKYLYEIARRHPYFYAPELLFFAKRYKAAFTECCQAADKAACLLPKLDELRDEGKASSAKQRLKCASLQKFGERAFKAWAVARLSQRFPKAEFAEVSKLVTDLTKVHTECCHGDLLECADDRADLAKYICENQDSISSKLKECCEKPLLEKSHCIAEVENDEMPADLPSLAADFVESKDVCKNYAEAKDVFLGMFLYEYARRHPDYSVVLLLRLAKTYETTLEKCCAAADPHECYAKVFDEFKPLVEEPQNLIKQNCELFEQLGEYKFQNALLVRYTKKVPQVSTPTLVEVSRNLGKVGSKCCKHPEAKRMPCAEDYLSVVLNQLCVLHEKTPVSDRVTKCCTESLVNRRPCFSALEVDETYVPKEFNAETFTFHADICTLSEKERQIKKQTALVELVKHKPKATKEQLKAVMDDFAAFVEKCCKADDKETCFAEEGKKLVAASQAALGLFPTIPLSRLFDNAMLRAHRLHQLAFDTYQEFEEAYIPKEQKYSFLQNPQTSLCFSESIPTPSNREETQQKSNLELLRISLLLIQSWLEPVQFLRSVFANSLVYGASDSNVYDLLKDLEEGIQTLMGRLEDGSPRTGQIFKQTYSKFDTNSHNDDALLKNYGLLYCFRKDMDKVETFLRIVQCRSVEGSCGF

SEQ ID NO: 33 - DNA, 2421 bp, Artificial Sequence
  Sequence containing HSA-22KhGH gene, synthetic
acgcgtcaccatgaagtgggtaacctttatttcccttctttttctctttagctcggcttattccaggggtgtgtttcgtcgagatgcacacaagagtgaggttgctcatcggtttaaagatttgggagaagaaaatttcaaagccttggtgttgattgcctttgctcagtatcttcagcagtgtccatttgaagatcatgtaaaattagtgaatgaagtaactgaatttgcaaaaacatgtgttgctgatgagtcagctgaaaattgtgacaaatcacttcataccctttttggagacaaattatgcacagttgcaactcttcgtgaaacctatggtgaaatggctgactgctgtgcaaaacaagaacctgagagaaatgaatgcttcttgcaacacaaagatgacaacccaaacctcccccgattggtgagaccagaggttgatgtgatgtgcactgcttttcatgacaatgaagagacatttttgaaaaaatacttatatgaaattgccagaagacatccttacttttatgccccggaactccttttctttgctaaaaggtataaagctgcttttacagaatgttgccaagctgctgataaagctgcctgcctgttgccaaagctcgatgaacttcgggatgaagggaaggcttcgtctgccaaacagagactcaagtgtgccagtctccaaaaatttggagaaagagctttcaaagcatgggcagtagctcgcctgagccagagatttcccaaagctgagtttgcagaagtttccaagttagtgacagatcttaccaaagtccacacggaatgctgccatggagatctgcttgaatgtgctgatgacagggcggaccttgccaagtatatctgtgaaaatcaagattcgatctccagtaaactgaaggaatgctgtgaaaaacctctgttggaaaaatcccactgcattgccgaagtggaaaatgatgagatgcctgctgacttgccttcattagctgctgattttgttgaaagtaaggatgtttgcaaaaactatgctgaggcaaaggatgtcttcctgggcatgtttttgtatgaatatgcaagaaggcatcctgattactctgtcgtgctgctgctgagacttgccaagacatatgaaaccactctagagaagtgctgtgccgctgcagatcctcatgaatgctatgccaaagtgttcgatgaatttaaacctcttgtggaagagcctcagaatttaatcaaacaaaattgtgagctttttgagcagcttggagagtacaaattccagaatgcgctattagttcgttacaccaagaaagtaccccaagtgtcaactccaactcttgtagaggtctcaagaaacctaggaaaagtgggcagcaaatgttgtaaacatcctgaagcaaaaagaatgccctgtgcagaagactatctatccgtggtcctgaaccagttatgtgtgttgcatgagaaaacgccagtaagtgacagagtcaccaaatgctgcacagaatccttggtgaacaggcgaccatgcttttcagctctggaagtcgatgaaacatacgttcccaaagagtttaatgctgaaacattcaccttccatgcagatatatgcacactttctgagaaggagagacaaatcaagaaacaaactgcacttgttgagctcgtgaaacacaagcccaaggcaacaaaagagcaactgaaagctgttatggatgatttcgcagcttttgtagagaagtgctgcaaggctgacgataaggagacctgctttgccgaggagggtaaaaaacttgttgctgcaagtcaagctgccttaggcttattcccaaccattcccttatccaggctttttgacaacgctatgctccgcgcccatcgtctgcaccagctggcctttgacacctaccaggagtttgaagaagcctatatcccaaaggaacagaagtattcattcctgcagaacccccagacctccctctgtttctcagagtctattccgacaccctccaacagggaggaaacacaacagaaatccaacctagagctgctccgcatctccctgctgctcatccagtcgtggctggagcccgtgcagttcctcaggagtgtcttcgccaacagcctggtgtacggcgcctctgacagcaacgtctatgacctcctaaaggacctagaggaaggcatccaaacgctgatggggaggctggaagatggcagcccccggactgggcagatcttcaagcagacctacagcaagttcgacacaaactcacacaacgatgacgcactactcaagaactacgggctgctctactgcttcaggaaggacatggacaaggtcgagacattcctgcgcatcgtgcagtgccgctctgtggagggcagctgtggcttctaagcggccgc

SEQ ID NO: 34 - protein, 776 aa, Artificial Sequence
  mHSA-22KhGH
DAHKSEVAHRFKDLGEENFKALVLIAFAQYLQQCPFEDHVKLVNEVTEFAKTCVADESAENCDKSLHTLFGDKLCTVATLRETYGEMADCCAKQEPERNECFLQHKDDNPNLPRLVRPEVDVMCTAFHDNEETFLKKYLYEIARRHPYFYAPELLFFAKRYKAAFTECCQAADKAACLLPKLDELRDEGKASSAKQRLKCASLQKFGERAFKAWAVARLSQRFPKAEFAEVSKLVTDLTKVHTECCHGDLLECADDRADLAKYICENQDSISSKLKECCEKPLLEKSHCIAEVENDEMPADLPSLAADFVESKDVCKNYTEAKDVFLGMFLYEYARRHPDYSVVLLLRLAKTYETTLEKCCAAADPHECYAKVFDEFKPLVEEPQNLIKQNCELFEQLGEYKFQNALLVRYTKKVPQVSTPTLVEVSRNLGKVGSKCCKHPEAKRMPCAEDYLSVVLNQLCVLHEKTPVSDRVTKCCTESLVNRRPCFSALEVDETYVPKEFNAETFTFHADICTLSEKERQIKKQTALVELVKHKPKATKEQLKAVMDDFAAFVEKCCKADDKETCFAEEGKKLVAASQAALGLFPTIPLSRLFDNAMLRAHRLHQLAFDTYQEFEEAYIPKEQKYSFLQNPQTSLCFSESIPTPSNREETQQKSNLELLRISLLLIQSWLEPVQFLRSVFANSLVYGASDSNVYDLLKDLEEGIQTLMGRLEDGSPRTGQIFKQTYSKFDTNSHNDDALLKNYGLLYCFRKDMDKVETFLRIVQCRSVEGSCGF

SEQ ID NO: 35 - DNA, 27 bp, Artificial Sequence
  Primer YA082, synthetic
aactatactgaggcaaaggatgtcttc

SEQ ID NO: 36 - DNA, 27 bp, Artificial Sequence
  Primer YA083, synthetic
tgcctcagtatagtttttgcaaacatc

SEQ ID NO: 37 - protein, 776 aa, Artificial Sequence
  22KhGH-HSA, mature
FPTIPLSRLFDNAMLRAHRLHQLAFDTYQEFEEAYIPKEQKYSFLQNPQTSLCFSESIPTPSNREETQQKSNLELLRISLLLIQSWLEPVQFLRSVFANSLVYGASDSNVYDLLKDLEEGIQTLMGRLEDGSPRTGQIFKQTYSKFDTNSHNDDALLKNYGLLYCFRKDMDKVETFLRIVQCRSVEGSCGFDAHKSEVAHRFKDLGEENFKALVLIAFAQYLQQCPFEDHVKLVNEVTEFAKTCVADESAENCDKSLHTLFGDKLCTVATLRETYGEMADCCAKQEPERNECFLQHKDDNPNLPRLVRPEVDVMCTAFHDNEETFLKKYLYEIARRHPYFYAPELLFFAKRYKAAFTECCQAADKAACLLPKLDELRDEGKASSAKQRLKCASLQKFGERAFKAWAVARLSQRFPKAEFAEVSKLVTDLTKVHTECCHGDLLECADDRADLAKYICENQDSISSKLKECCEKPLLEKSHCIAEVENDEMPADLPSLAADFVESKDVCKNYAEAKDVFLGMFLYEYARRHPDYSVVLLLRLAKTYETTLEKCCAAADPHECYAKVFDEFKPLVEEPQNLIKQNCELFEQLGEYKFQNALLVRYTKKVPQVSTPTLVEVSRNLGKVGSKCCKHPEAKRMPCAEDYLSVVLNQLCVLHEKTPVSDRVTKCCTESLVNRRPCFSALEVDETYVPKEFNAETFTFHADICTLSEKERQIKKQTALVELVKHKPKATKEQLKAVMDDFAAFVEKCCKADDKETCFAEEGKKLVAASQAALGL

SEQ ID NO: 38 - DNA, 2427 bp, Artificial Sequence
  Sequence containing 22KhGH-HSA gene, synthetic
acgcgtcaccatggctacaggctcccggacgtccctgctcctggcttttggcctgctctgcctgccctggcttcaagagggcagtgccttcccaaccattcccttatccaggctttttgacaacgctatgctccgcgcccatcgtctgcaccagctggcctttgacacctaccaggagtttgaagaagcctatatcccaaaggaacagaagtattcattcctgcagaacccccagacctccctctgtttctcagagtctattccgacaccctccaacagggaggaaacacaacagaaatccaacctagagctgctccgcatctccctgctgctcatccagtcgtggctggagcccgtgcagttcctcaggagtgtcttcgccaacagcctggtgtacggcgcctctgacagcaacgtctatgacctcctaaaggacctagaggaaggcatccaaacgctgatggggaggctggaagatggcagcccccggactgggcagatcttcaagcagacctacagcaagttcgacacaaactcacacaacgatgacgcactactcaagaactacgggctgctctactgcttcaggaaggacatggacaaggtcgagacattcctgcgcatcgtgcagtgccgctctgtggagggcagctgtggcttcgatgcacacaagagtgaggttgctcatcggtttaaagatttgggagaagaaaatttcaaagccttggtgttgattgcctttgctcagtatcttcagcagtgtccatttgaagatcatgtaaaattagtgaatgaagtaactgaatttgcaaaaacatgtgttgctgatgagtcagctgaaaattgtgacaaatcacttcataccctttttggagacaaattatgcacagttgcaactcttcgtgaaacctatggtgaaatggctgactgctgtgcaaaacaagaacctgagagaaatgaatgcttcttgcaacacaaagatgacaacccaaacctcccccgattggtgagaccagaggttgatgtgatgtgcactgcttttcatgacaatgaagagacatttttgaaaaaatacttatatgaaattgccagaagacatccttacttttatgccccggaactccttttctttgctaaaaggtataaagctgcttttacagaatgttgccaagctgctgataaagctgcctgcctgttgccaaagctcgatgaacttcgggatgaagggaaggcttcgtctgccaaacagagactcaagtgtgccagtctccaaaaatttggagaaagagctttcaaagcatgggcagtagctcgcctgagccagagatttcccaaagctgagtttgcagaagtttccaagttagtgacagatcttaccaaagtccacacggaatgctgccatggagatctgcttgaatgtgctgatgacagggcggaccttgccaagtatatctgtgaaaatcaagattcgatctccagtaaactgaaggaatgctgtgaaaaacctctgttggaaaaatcccactgcattgccgaagtggaaaatgatgagatgcctgctgacttgccttcattagctgctgattttgttgaaagtaaggatgtttgcaaaaactatgctgaggcaaaggatgtcttcctgggcatgtttttgtatgaatatgcaagaaggcatcctgattactctgtcgtgctgctgctgagacttgccaagacatatgaaaccactctagagaagtgctgtgccgctgcagatcctcatgaatgctatgccaaagtgttcgatgaatttaaacctcttgtggaagagcctcagaatttaatcaaacaaaattgtgagctttttgagcagcttggagagtacaaattccagaatgcgctattagttcgttacaccaagaaagtaccccaagtgtcaactccaactcttgtagaggtctcaagaaacctaggaaaagtgggcagcaaatgttgtaaacatcctgaagcaaaaagaatgccctgtgcagaagactatctatccgtggtcctgaaccagttatgtgtgttgcatgagaaaacgccagtaagtgacagagtcaccaaatgctgcacagaatccttggtgaacaggcgaccatgcttttcagctctggaagtcgatgaaacatacgttcccaaagagtttaatgctgaaacattcaccttccatgcagatatatgcacactttctgagaaggagagacaaatcaagaaacaaactgcacttgttgagctcgtgaaacacaagcccaaggcaacaaaagagcaactgaaagctgttatggatgatttcgcagcttttgtagagaagtgctgcaaggctgacgataaggagacctgctttgccgaggagggtaaaaaacttgttgctgcaagtcaagctgccttaggcttataagcggccgc

SEQ ID NO: 39 - protein, 776 aa, Artificial Sequence; identical to SEQ ID NO: 11
  22KhGH-mHSA, mature

SEQ ID NO: 40 - DNA, 792 bp, Artificial Sequence
  Sequence coding synthetic hGHR ECD gene
atggacctgtggcagctcctcctgaccctcgctctggctggctcctccgatgccttctccggctccgaggccaccgctgctatcctgagcagggctccctggtccctgcagagcgtcaaccctggcctgaagaccaactcctccaaagagcccaagttcacaaagtgcaggtcccccgagagggagaccttctcctgtcattggaccgacgaggtgcaccacggcaccaagaacctgggccccatccagctcttctacaccaggaggaacacccaagagtggacacaggagtggaaggagtgccccgattacgtgtccgccggcgagaacagctgctacttcaactcctccttcacatccatctggattccttattgcatcaaactgacctccaacggcggcacagtggatgagaagtgcttcagcgtcgacgagatcgtgcagcccgatccccccatcgctctgaactggaccctgctgaatgtgtccctgaccggcatccacgccgatattcaggtgaggtgggaggctcccaggaacgctgacatccagaagggctggatggtcctggagtacgagctgcagtacaaggaggtcaacgagaccaagtggaaaatgatggaccctatcctgacaacatccgtccctgtgtacagcctgaaggtggacaaagagtacgaggtgagggtgaggagcaaacagcggaatagcggcaactacggagaattctccgaggtgctgtatgtgaccctgccccagatgtcccagttcacctgtgaagaggacttttac

SEQ ID NO: 41 - DNA, 42 bp, Artificial Sequence
  Primer YA034, synthetic
ccgacgcgtcgccaccatggacctgtggcagctcctcctgac

SEQ ID NO: 42 - DNA, 67 bp, Artificial Sequence
  Primer YA035, synthetic
cactgttagcccgaatattccgaagatgataattaggagccatgggaagtaaaagtcctcttcacag

SEQ ID NO: 43 - DNA, 43 bp, Artificial Sequence
  Primer K708, synthetic
ccggtcgaccgccaccatggatctctggcagctgctgttgacc

SEQ ID NO: 44 - DNA, 39 bp, Artificial Sequence
  Primer K709, synthetic
tttggcggccgcctaaggcatgattttgttcagttggtc

SEQ ID NO: 45 - DNA, 1917 bp, Artificial Sequence
  Sequence coding synthetic hGHR gene
atggacctgtggcagctcctcctgaccctcgctctggctggctcctccgatgccttctccggctccgaggccaccgctgctatcctgagcagggctccctggtccctgcagagcgtcaaccctggcctgaagaccaactcctccaaagagcccaagttcacaaagtgcaggtcccccgagagggagaccttctcctgtcattggaccgacgaggtgcaccacggcaccaagaacctgggccccatccagctcttctacaccaggaggaacacccaagagtggacacaggagtggaaggagtgccccgattacgtgtccgccggcgagaacagctgctacttcaactcctccttcacatccatctggattccttattgcatcaaactgacctccaacggcggcacagtggatgagaagtgcttcagcgtcgacgagatcgtgcagcccgatccccccatcgctctgaactggaccctgctgaatgtgtccctgaccggcatccacgccgatattcaggtgaggtgggaggctcccaggaacgctgacatccagaagggctggatggtcctggagtacgagctgcagtacaaggaggtcaacgagaccaagtggaaaatgatggaccctatcctgacaacatccgtccctgtgtacagcctgaaggtggacaaagagtacgaggtgagggtgaggagcaaacagcggaatagcggcaactacggagaattctccgaggtgctgtatgtgaccctgccccagatgtcccagttcacctgtgaagaggacttttacttcccatggctcctaattatcatcttcggaatattcgggctaacagtgatgctatttgtattcttattttctaaacagcaaaggattaaaatgctgattctgcccccagttccagttccaaagattaaaggaatcgatccagatctcctcaaggaaggaaaattagaggaggtgaacacaatcttagccattcatgatagctataaacccgaattccacagtgatgactcttgggttgaatttattgagctagatattgatgagccagatgaaaagactgaggaatcagacacagacagacttctaagcagtgaccatgagaaatcacatagtaacctaggggtgaaggatggcgactctggacgtaccagctgttgtgaacctgacattctggagactgatttcaatgccaatgacatacatgagggtacctcagaggttgctcagccacagaggttaaaaggggaagcagatctcttatgccttgaccagaagaatcaaaataactcaccttatcatgatgcttgccctgctactcagcagcccagtgttatccaagcagagaaaaacaaaccacaaccacttcctactgaaggagctgagtcaactcaccaagctgcccatattcagctaagcaatccaagttcactgtcaaacatcgacttttatgcccaggtgagcgacattacaccagcaggtagtgtggtcctttccccgggccaaaagaataaggcagggatgtcccaatgtgacatgcacccggaaatggtctcactctgccaagaaaacttccttatggacaatgcctacttctgtgaggcagatgccaaaaagtgcatccctgtggctcctcacatcaaggttgaatcacacatacagccaagcttaaaccaagaggacatttacatcaccacagaaagccttaccactgctgctgggaggcctgggacaggagaacatgttccaggttctgagatgcctgtcccagactatacctccattcatatagtacagtccccacagggcctcatactcaatgcgactgccttgcccttgcctgacaaagagtttctctcatcatgtggctatgtgagcacagaccaactgaacaaaatcatgccttag